European Patent Specification EP 3 908 673 B1, published December 11, 2024. Title: COMPOSITIONS AND METHODS FOR CHROMATIN AND GENE EXPRESSION ANALYSIS IN SINGLE CELLS. Applicant: Agilent Technologies, Inc. The Trustees Of The University of Pennsylvania. Application not yet assigned. The sequence listing filed with the application follows.

SEQUENCE LISTING (19 sequences)

SEQ ID NO: 1 - DNA, 63 bp, Artificial Sequence
  Synthetic oligonucleotide
  N_region (45)..(59): n is any nucleotide
  misc_feature (45)..(59): n is a, c, g, or t
ggagaattgtaatacgactcactatagggagacgcgtgatcacgnnnnnnnnnnnnnnntgtg

SEQ ID NO: 2 - DNA, 60 bp, Artificial Sequence
  Synthetic oligonucleotide
  N_region (45)..(59): n is any nucleotide
  misc_feature (45)..(59): n is a, c, g, or t
ggagaattgtaatacgactcactatagggagacgcgtgatcacgnnnnnnnnnnnnnnnt

SEQ ID NO: 3 - DNA, 62 bp, Artificial Sequence
  Synthetic oligonucleotide
  N_region (4)..(18): n is any nucleotide
  misc_feature (4)..(18): n is a, c, g, or t
aaannnnnnnnnnnnnnncgtgatcacgcgtctccctatagtgagtcgtattacaattctcc

SEQ ID NO: 4 - DNA, 47 bp, Artificial Sequence
  Synthetic oligonucleotide
ggagaattgtaatacgactcactatagggagacgcgtgatcacgaca

SEQ ID NO: 5 - DNA, 44 bp, Artificial Sequence
  Synthetic oligonucleotide
cgtgatcacgcgtctccctatagtgagtcgtattacaattctcc

SEQ ID NO: 6 - DNA, 23 bp, Artificial Sequence
  Synthetic oligonucleotide
  N_region (8)..(22): n is any nucleotide
  misc_feature (8)..(22): n is a, c, g, or t
atgaggannnnnnnnnnnnnnnt

SEQ ID NO: 7 - DNA, 28 bp, Artificial Sequence
  Synthetic oligonucleotide
  N_region (4)..(18): n is any nucleotide
  misc_feature (4)..(18): n is a, c, g, or t
aaannnnnnnnnnnnnnntcctcattgt

SEQ ID NO: 8 - DNA, 18 bp, Artificial Sequence
  Synthetic oligonucleotide
tagggagacgcgtgatca

SEQ ID NO: 9 - DNA, 18 bp, Artificial Sequence
  Synthetic oligonucleotide
tagggagacgcgtgagtt

SEQ ID NO: 10 - DNA, 34 bp, Artificial Sequence
  Synthetic oligonucleotide
gcgccattgaccaggattttcccccccccccccc

SEQ ID NO: 11 - DNA, 21 bp, Artificial Sequence
  Synthetic oligonucleotide
gcgccattgaccaggattttc

SEQ ID NO: 12 - DNA, 20 bp, Artificial Sequence
  Synthetic oligonucleotide
tccttagctgttgcagaaat

SEQ ID NO: 13 - DNA, 20 bp, Artificial Sequence
  Synthetic oligonucleotide
cgttcagttgatgcagagtg

SEQ ID NO: 14 - DNA, 20 bp, Artificial Sequence
  Synthetic oligonucleotide
agaagcagcttcaaacctgc

SEQ ID NO: 15 - DNA, 20 bp, Artificial Sequence
  Synthetic oligonucleotide
aagttagctttacagtgggc

SEQ ID NO: 16 - DNA, 20 bp, Artificial Sequence
  Synthetic oligonucleotide
ggtgttggttctcttaatct

SEQ ID NO: 17 - DNA, 20 bp, Artificial Sequence
  Synthetic oligonucleotide
atttagttggggcatttcac

SEQ ID NO: 18 - DNA, 20 bp, Artificial Sequence
  Synthetic oligonucleotide
ttatggtgggtcatacggta

SEQ ID NO: 19 - DNA, 20 bp, Artificial Sequence
  Synthetic oligonucleotide
tagtgtaaggagtatggggg